European Patent Application EP 4 559 478 A1, published May 28, 2025. Title: Method for Reducing Pyrogenic Activity of Inactivated Whole Particle Influenza Vaccine. Applicant: Denka Company Limited. The sequence listing filed with the application follows.

SEQUENCE LISTING (5 sequences)

SEQ ID NO: 1 - RNA, 25 nt, Gallus gallus
  source 1..25: mol_type = genomic RNA
agctggtttcatatggtggtttaga

SEQ ID NO: 2 - RNA, 22 nt, Gallus gallus
  source 1..22: mol_type = genomic RNA
aagctgccagttgaagaactgt

SEQ ID NO: 3 - RNA, 24 nt, Gallus gallus
  source 1..24: mol_type = genomic RNA
gcgctcaggctggtgctgggggat

SEQ ID NO: 4 - RNA, 22 nt, Gallus gallus
  source 1..22: mol_type = genomic RNA
ttaatgctaatcgtgatagggg

SEQ ID NO: 5 - RNA, 23 nt, Gallus gallus
  source 1..23: mol_type = genomic RNA
gaaatcaagggtgggtaagacct